European Patent Application EP 4 574 817 A1, published June 25, 2025. Title: INHIBITORY COMPOUNDS. Applicant: LoQus23 Therapeutics Limited. Application EP. The sequence listing filed with the application follows.

SEQUENCE LISTING (3 sequences)

SEQ ID NO: 1 - DNA, 25 bp, synthetic construct
  source 1..25: mol_type = other DNA; note = CAG Looped DNA sequence
tcatcgatcgcaggcttcagatagg

SEQ ID NO: 2 - DNA, 24 bp, synthetic construct
  source 1..24: mol_type = other DNA; note = CAG Looped DNA sequence
cctctatctgaagccgatcgatgg

SEQ ID NO: 3 - DNA, 7406 bp, synthetic construct
  source 1..7406: mol_type = other DNA; note = pcDNA4/TO-100CAG (7160bp) Vector
gatgtacgggccagatatacgcgttgacattgattattgactagttattaatagtaatcaattacggggtcattagttcatagcccatatatggagttccgcgttacataacttacggtaaatggcccgcctggctgaccgcccaacgacccccgcccattgacgtcaataatgacgtatgttcccatagtaacgccaatagggactttccattgacgtcaatgggtggagtatttacggtaaactgcccacttggcagtacatcaagtgtatcatatgccaagtacgccccctattgacgtcaatgacggtaaatggcccgcctggcattatgcccagtacatgaccttatgggactttcctacttggcagtacatctacgtattagtcatcgctattaccatggtgatgcggttttggcagtacatcaatgggcgtggatagcggtttgactcacggggatttccaagtctccaccccattgacgtcaatgggagtttgttttggaaccaaaatcaacgggactttccaaaatgtcgtaacaactccgccccattgacgcaaatgggcggtaggcgtgtacggtgggaggtctatataagcagagctctccctatcagtgatagagatctccctatcagtgatagagatcgtcgacgagctcgtttagtgaaccgtcagatcgcctggagacgccatccacgctgttttgacctccatagaagacaccgggaccgatccagcctccggactctagcgtttaaacttaagcttaccatggcgaccctggaaaagctgatgaaggccttcgagtccctcaagtccttccagcagcagcagcagcagcagcagcagcagcagcagcagcagcagcagcagcagcagcagcagcagcagcagcagcagcagcagcagcagcagcagcagcagcagcagcagcagcagcagcagcagcagcagcagcagcagcagcagcagcagcagcagcagcagcagcagcagcagcagcagcagcagcagcagcagcagcagcagcagcagcagcagcagcagcagcagcagcagcagcagcagcagcagcagcagcagcagcagcagcagcagcagcagcagcagcagcagcagcagcaacagccgccaccgccgccgccgccgccgccgcctcctcagcttcctcagccgccgccgcaggcacagccgctgctgcctcagccgcagccgcccccgccgccgcccccgccgccacccggcccggctgtggctgaggagccgctgcaccgaccaggtaccggcagcggcgccacaaacttctctctgctaaagcaagcaggtgatgttgaagaaaaccccgggcctggatccatggtcttcacactcgaagatttcgttggggactggcgacagacagccggctacaacctggaccaagtccttgaacagggaggtgtgtccagtttgtttcagaatctcggggtgtccgtaactccgatccaaaggattgtcctgagcggtgaaaatgggctgaagatcgacatccatgtcatcatcccgtatgaaggtctgagcggcgaccaaatgggccagatcgaaaaaatttttaaggtggtgtaccctgtggatgatcatcactttaaggtgatcctgcactatggcacactggtaatcgacggggttacgccgaacatgatcgactatttcggacggccgtatgaaggcatcgccgtgttcgacggcaaaaagatcactgtaacagggaccctgtggaacggcaacaaaattatcgacgagcgcctgatcaaccccgacggctccctgctgttccgagtaaccatcaacggagtgaccggctggcggctgtgcgaacgcattctggcgtaagaattccggcaataaaaagacagaataaaacgcacggtgttgggtcgtttgttccgttacataacttacggtaaatggcccgcctggctgaccgcccaacgacccccgcccattgacgtcaataatgacgtatgttcccatagtaacgccaatagggactttccattgacgtcaatgggtggagtatttacggtaaactgcccacttggcagtacatcaagtgtatcatatgccaagtacgccccctattgacgtcaatgacggtaaatggcccgcctggcattatgcccagtacatgaccttatgggactttcctacttggcagtacatctacgtattagtcatcgctattaccatggtgatgcggttttggcagtacatcaatgggcgtggatagcggtttgactcacggggatttccaagtctccaccccattgacgtcaatgggagtttgttttggcaccaaaatcaacgggactttccaaaatgtcgtaacaactccgccccattgacgcaaatgggcggtaggcgtgtacggtgggaggtctatataagcagagctatcgatgccaccatggtgagcaagggcgaggagctgttcaccggggtggtgcccatcctggtcgagctggacggcgacgtaaacggccacaagttcagcgtgtccggcgagggcgagggcgatgccacctacggcaagctgaccctgaagttcatctgcaccaccggcaagctgcccgtgccctggcccaccctcgtgaccaccctgacctacggcgtgcagtgcttcagccgctaccccgaccacatgaagcagcacgacttcttcaagtccgccatgcccgaaggctacgtccaggagcgcaccatcttcttcaaggacgacggcaactacaagacccgcgccgaggtgaagttcgagggcgacaccctggtgaaccgcatcgagctgaagggcatcgacttcaaggaggacggcaacatcctggggcacaagctggagtacaactacaacagccacaacgtctatatcatggccgacaagcagaagaacggcatcaaggtgaacttcaagatccgccacaacatcgaggacggcagcgtgcagctcgccgaccactaccagcagaacacccccatcggcgacggccccgtgctgctgcccgacaaccactacctgagcacccagtccgccctgagcaaagaccccaacgagaagcgcgatcacatggtcctgctggagttcgtgaccgccgccgggatcactctcggcatggacgagctgtacaaggctcgagtctagagggcccgtttaaacccgctgatcagcctcgactgtgccttctagttgccagccatctgttgtttgcccctcccccgtgccttccttgaccctggaaggtgccactcccactgtcctttcctaataaaatgaggaaattgcatcgcattgtctgagtaggtgtcattctattctggggggtggggtggggcaggacagcaagggggaggattgggaagacaatagcaggcatgctggggatgcggtgggctctatggcttctgaggcggaaagaaccagctggggctctagggggtatccccacgcgccctgtagcggcgcattaagcgcggcgggtgtggtggttacgcgcagcgtgaccgctacacttgccagcgccctagcgcccgctcctttcgctttcttcccttcctttctcgccacgttcgccggctttccccgtcaagctctaaatcgggggctccctttagggttccgatttagtgctttacggcacctcgaccccaaaaaacttgattagggtgatggttcacgtagtgggccatcgccctgatagacggtttttcgccctttgacgttggagtccacgttctttaatagtggactcttgttccaaactggaacaacactcaaccctatctcggtctattcttttgatttataagggattttgccgatttcggcctattggttaaaaaatgagctgatttaacaaaaatttaacgcgaattaattctgtggaatgtgtgtcagttagggtgtggaaagtccccaggctccccagcaggcagaagtatgcaaagcatgcatctcaattagtcagcaaccaggtgtggaaagtccccaggctccccagcaggcagaagtatgcaaagcatgcatctcaattagtcagcaaccatagtcccgcccctaactccgcccatcccgcccctaactccgcccagttccgcccattctccgccccatggctgactaattttttttatttatgcagaggccgaggccgcctctgcctctgagctattccagaagtagtgaggaggcttttttggaggcctaggcttttgcaaaaagctcccgggagcttgtatatccattttcggatctgatcagcacgtgttgacaattaatcatcggcatagtatatcggcatagtataatacgacaaggtgaggaactaaaccatggccaagttgaccagtgccgttccggtgctcaccgcgcgcgacgtcgccggagcggtcgagttctggaccgaccggctcgggttctcccgggacttcgtggaggacgacttcgccggtgtggtccgggacgacgtgaccctgttcatcagcgcggtccaggaccaggtggtgccggacaacaccctggcctgggtgtgggtgcgcggcctggacgagctgtacgccgagtggtcggaggtcgtgtccacgaacttccgggacgcctccgggccggccatgaccgagatcggcgagcagccgtgggggcgggagttcgccctgcgcgacccggccggcaactgcgtgcacttcgtggccgaggagcaggactgacacgtgctacgagatttcgattccaccgccgccttctatgaaaggttgggcttcggaatcgttttccgggacgccggctggatgatcctccagcgcggggatctcatgctggagttcttcgcccaccccaacttgtttattgcagcttataatggttacaaataaagcaatagcatcacaaatttcacaaataaagcatttttttcactgcattctagttgtggtttgtccaaactcatcaatgtatcttatcatgtctgtataccgtcgacctctagctagagcttggcgtaatcatggtcatagctgtttcctgtgtgaaattgttatccgctcacaattccacacaacatacgagccggaagcataaagtgtaaagcctggggtgcctaatgagtgagctaactcacattaattgcgttgcgctcactgcccgctttccagtcgggaaacctgtcgtgccagctgcattaatgaatcggccaacgcgcggggagaggcggtttgcgtattgggcgctcttccgcttcctcgctcactgactcgctgcgctcggtcgttcggctgcggcgagcggtatcagctcactcaaaggcggtaatacggttatccacagaatcaggggataacgcaggaaagaacatgtgagcaaaaggccagcaaaaggccaggaaccgtaaaaaggccgcgttgctggcgtttttccataggctccgcccccctgacgagcatcacaaaaatcgacgctcaagtcagaggtggcgaaacccgacaggactataaagataccaggcgtttccccctggaagctccctcgtgcgctctcctgttccgaccctgccgcttaccggatacctgtccgcctttctcccttcgggaagcgtggcgctttctcatagctcacgctgtaggtatctcagttcggtgtaggtcgttcgctccaagctgggctgtgtgcacgaaccccccgttcagcccgaccgctgcgccttatccggtaactatcgtcttgagtccaacccggtaagacacgacttatcgccactggcagcagccactggtaacaggattagcagagcgaggtatgtaggcggtgctacagagttcttgaagtggtggcctaactacggctacactagaagaacagtatttggtatctgcgctctgctgaagccagttaccttcggaaaaagagttggtagctcttgatccggcaaacaaaccaccgctggtagcggtttttttgtttgcaagcagcagattacgcgcagaaaaaaaggatctcaagaagatcctttgatcttttctacggggtctgacgctcagtggaacgaaaactcacgttaagggattttggtcatgagattatcaaaaaggatcttcacctagatccttttaaattaaaaatgaagttttaaatcaatctaaagtatatatgagtaaacttggtctgacagttaccaatgcttaatcagtgaggcacctatctcagcgatctgtctatttcgttcatccatagttgcctgactccccgtcgtgtagataactacgatacgggagggcttaccatctggccccagtgctgcaatgataccgcgagacccacgctcaccggctccagatttatcagcaataaaccagccagccggaagggccgagcgcagaagtggtcctgcaactttatccgcctccatccagtctattaattgttgccgggaagctagagtaagtagttcgccagttaatagtttgcgcaacgttgttgccattgctacaggcatcgtggtgtcacgctcgtcgtttggtatggcttcattcagctccggttcccaacgatcaaggcgagttacatgatcccccatgttgtgcaaaaaagcggttagctccttcggtcctccgatcgttgtcagaagtaagttggccgcagtgttatcactcatggttatggcagcactgcataattctcttactgtcatgccatccgtaagatgcttttctgtgactggtgagtactcaaccaagtcattctgagaatagtgtatgcggcgaccgagttgctcttgcccggcgtcaatacgggataataccgcgccacatagcagaactttaaaagtgctcatcattggaaaacgttcttcggggcgaaaactctcaaggatcttaccgctgttgagatccagttcgatgtaacccactcgtgcacccaactgatcttcagcatcttttactttcaccagcgtttctgggtgagcaaaaacaggaaggcaaaatgccgcaaaaaagggaataagggcgacacggaaatgttgaatactcatactcttcctttttcaatattattgaagcatttatcagggttattgtctcatgagcggatacatatttgaatgtatttagaaaaataaacaaataggggttccgcgcacatttccccgaaaagtgccacctgacgtcgacggatcgggagatctcccgatcccctatggtgcactctcagtacaatctgctctgatgccgcatagttaagccagtatctgctccctgcttgtgtgttggaggtcgctgagtagtgcgcgagcaaaatttaagctacaacaaggcaaggcttgaccgacaattgcatgaagaatctgcttagggttaggcgttttgcgctgcttcgc